European Patent Specification EP 3 998 343 B1, published March 20, 2024. Title: Library-tag composition and uses thereof in MGI sequencing platform. Applicant: Nanodigmbio (Nanjing) Biotechnology Co., Ltd. The sequence listing filed with the application follows.

SEQUENCE LISTING (798 sequences)

SEQ ID NO: 1 - DNA, 10 bp, Artificial Sequence
  tag sequence for base balance
tcacattgct

SEQ ID NO: 2 - DNA, 10 bp, Artificial Sequence
  tag sequence for base balance
aatggcgctc

SEQ ID NO: 3 - DNA, 10 bp, Artificial Sequence
  tag sequence for base balance
gtctcaatga

SEQ ID NO: 4 - DNA, 10 bp, Artificial Sequence
  tag sequence for base balance
cggatgcaag

SEQ ID NO: 5 - DNA, 10 bp, Artificial Sequence
  tag sequence for base balance
tcgcttaagc

SEQ ID NO: 6 - DNA, 10 bp, Artificial Sequence
  tag sequence for base balance
cgaggcttag

SEQ ID NO: 7 - DNA, 10 bp, Artificial Sequence
  tag sequence for base balance
gtctaaggct

SEQ ID NO: 8 - DNA, 10 bp, Artificial Sequence
  tag sequence for base balance
aatacgccta

SEQ ID NO: 9 - DNA, 10 bp, Artificial Sequence
  tag sequence for base balance
aagcctattg

SEQ ID NO: 10 - DNA, 10 bp, Artificial Sequence
  tag sequence for base balance
cgctactgca

SEQ ID NO: 11 - DNA, 10 bp, Artificial Sequence
  tag sequence for base balance
tcaagagcat

SEQ ID NO: 12 - DNA, 10 bp, Artificial Sequence
  tag sequence for base balance
gttgtgcagc

SEQ ID NO: 13 - DNA, 10 bp, Artificial Sequence
  tag sequence for base balance
agacaggaat

SEQ ID NO: 14 - DNA, 10 bp, Artificial Sequence
  tag sequence for base balance
ccttgccgta

SEQ ID NO: 15 - DNA, 10 bp, Artificial Sequence
  tag sequence for base balance
gtcattacgg

SEQ ID NO: 16 - DNA, 10 bp, Artificial Sequence
  tag sequence for base balance
taggcattcc

SEQ ID NO: 17 - DNA, 10 bp, Artificial Sequence
  tag sequence for base balance
catatcatcg

SEQ ID NO: 18 - DNA, 10 bp, Artificial Sequence
  tag sequence for base balance
gcacaacaat

SEQ ID NO: 19 - DNA, 10 bp, Artificial Sequence
  tag sequence for base balance
ttgtcgtggc

SEQ ID NO: 20 - DNA, 10 bp, Artificial Sequence
  tag sequence for base balance
agcggtgcta

SEQ ID NO: 21 - DNA, 10 bp, Artificial Sequence
  tag sequence for base balance
agccagtagg

SEQ ID NO: 22 - DNA, 10 bp, Artificial Sequence
  tag sequence for base balance
gtaagtgtac

SEQ ID NO: 23 - DNA, 10 bp, Artificial Sequence
  tag sequence for base balance
tagtcacgtt

SEQ ID NO: 24 - DNA, 10 bp, Artificial Sequence
  tag sequence for base balance
cctgtcacca

SEQ ID NO: 25 - DNA, 10 bp, Artificial Sequence
  tag sequence for base balance
atcgtggatg

SEQ ID NO: 26 - DNA, 10 bp, Artificial Sequence
  tag sequence for base balance
tggagatcga

SEQ ID NO: 27 - DNA, 10 bp, Artificial Sequence
  tag sequence for base balance
cctcacagat

SEQ ID NO: 28 - DNA, 10 bp, Artificial Sequence
  tag sequence for base balance
gaatctctcc

SEQ ID NO: 29 - DNA, 10 bp, Artificial Sequence
  tag sequence for base balance
gcagactgac

SEQ ID NO: 30 - DNA, 10 bp, Artificial Sequence
  tag sequence for base balance
ctcattaacg

SEQ ID NO: 31 - DNA, 10 bp, Artificial Sequence
  tag sequence for base balance
tggtgagctt

SEQ ID NO: 32 - DNA, 10 bp, Artificial Sequence
  tag sequence for base balance
aatccgctga

SEQ ID NO: 33 - DNA, 10 bp, Artificial Sequence
  tag sequence for base balance
tcgcatcaac

SEQ ID NO: 34 - DNA, 10 bp, Artificial Sequence
  tag sequence for base balance
agaacagtga

SEQ ID NO: 35 - DNA, 10 bp, Artificial Sequence
  tag sequence for base balance
catgtctcct

SEQ ID NO: 36 - DNA, 10 bp, Artificial Sequence
  tag sequence for base balance
gtctggagtg

SEQ ID NO: 37 - DNA, 10 bp, Artificial Sequence
  tag sequence for base balance
gaggtctgtg

SEQ ID NO: 38 - DNA, 10 bp, Artificial Sequence
  tag sequence for base balance
ctatagacgt

SEQ ID NO: 39 - DNA, 10 bp, Artificial Sequence
  tag sequence for base balance
tgcagtgacc

SEQ ID NO: 40 - DNA, 10 bp, Artificial Sequence
  tag sequence for base balance
actccactaa

SEQ ID NO: 41 - DNA, 10 bp, Artificial Sequence
  tag sequence for base balance
gcgaagtagg

SEQ ID NO: 42 - DNA, 10 bp, Artificial Sequence
  tag sequence for base balance
tgcctaacct

SEQ ID NO: 43 - DNA, 10 bp, Artificial Sequence
  tag sequence for base balance
aatggtctac

SEQ ID NO: 44 - DNA, 10 bp, Artificial Sequence
  tag sequence for base balance
ctatccggta

SEQ ID NO: 45 - DNA, 10 bp, Artificial Sequence
  tag sequence for base balance
tacgcttcag

SEQ ID NO: 46 - DNA, 10 bp, Artificial Sequence
  tag sequence for base balance
cggagcatct

SEQ ID NO: 47 - DNA, 10 bp, Artificial Sequence
  tag sequence for base balance
gtactagatc

SEQ ID NO: 48 - DNA, 10 bp, Artificial Sequence
  tag sequence for base balance
acttagcgga

SEQ ID NO: 49 - DNA, 10 bp, Artificial Sequence
  tag sequence for base balance
atcactccat

SEQ ID NO: 50 - DNA, 10 bp, Artificial Sequence
  tag sequence for base balance
gatcgcagtg

SEQ ID NO: 51 - DNA, 10 bp, Artificial Sequence
  tag sequence for base balance
ccggaattcc

SEQ ID NO: 52 - DNA, 10 bp, Artificial Sequence
  tag sequence for base balance
tgattggaga

SEQ ID NO: 53 - DNA, 10 bp, Artificial Sequence
  tag sequence for base balance
cacaaggtcg

SEQ ID NO: 54 - DNA, 10 bp, Artificial Sequence
  tag sequence for base balance
tctcgcagga

SEQ ID NO: 55 - DNA, 10 bp, Artificial Sequence
  tag sequence for base balance
gtggtatcat

SEQ ID NO: 56 - DNA, 10 bp, Artificial Sequence
  tag sequence for base balance
agatctcatc

SEQ ID NO: 57 - DNA, 10 bp, Artificial Sequence
  tag sequence for base balance
gatggagatt

SEQ ID NO: 58 - DNA, 10 bp, Artificial Sequence
  tag sequence for base balance
ctcattctgc

SEQ ID NO: 59 - DNA, 10 bp, Artificial Sequence
  tag sequence for base balance
tggcagacaa

SEQ ID NO: 60 - DNA, 10 bp, Artificial Sequence
  tag sequence for base balance
acatcctgcg

SEQ ID NO: 61 - DNA, 10 bp, Artificial Sequence
  tag sequence for base balance
acgtcgcaga

SEQ ID NO: 62 - DNA, 10 bp, Artificial Sequence
  tag sequence for base balance
tgtataggct

SEQ ID NO: 63 - DNA, 10 bp, Artificial Sequence
  tag sequence for base balance
caacacattg

SEQ ID NO: 64 - DNA, 10 bp, Artificial Sequence
  tag sequence for base balance
gtcggttcac

SEQ ID NO: 65 - DNA, 10 bp, Artificial Sequence
  tag sequence for base balance
agccataagc

SEQ ID NO: 66 - DNA, 10 bp, Artificial Sequence
  tag sequence for base balance
gtattccgag

SEQ ID NO: 67 - DNA, 10 bp, Artificial Sequence
  tag sequence for base balance
cataggttca

SEQ ID NO: 68 - DNA, 10 bp, Artificial Sequence
  tag sequence for base balance
tcggcagctt

SEQ ID NO: 69 - DNA, 10 bp, Artificial Sequence
  tag sequence for base balance
gttcggtcct

SEQ ID NO: 70 - DNA, 10 bp, Artificial Sequence
  tag sequence for base balance
tggattgtag

SEQ ID NO: 71 - DNA, 10 bp, Artificial Sequence
  tag sequence for base balance
ccagaacgtc

SEQ ID NO: 72 - DNA, 10 bp, Artificial Sequence
  tag sequence for base balance
aactccaaga

SEQ ID NO: 73 - DNA, 10 bp, Artificial Sequence
  tag sequence for base balance
cgtacactgg

SEQ ID NO: 74 - DNA, 10 bp, Artificial Sequence
  tag sequence for base balance
gcacacagca

SEQ ID NO: 75 - DNA, 10 bp, Artificial Sequence
  tag sequence for base balance
atggtgtatc

SEQ ID NO: 76 - DNA, 10 bp, Artificial Sequence
  tag sequence for base balance
tactgtgcat

SEQ ID NO: 77 - DNA, 10 bp, Artificial Sequence
  tag sequence for base balance
cggcaatcag

SEQ ID NO: 78 - DNA, 10 bp, Artificial Sequence
  tag sequence for base balance
gtagttcgga

SEQ ID NO: 79 - DNA, 10 bp, Artificial Sequence
  tag sequence for base balance
tacaggaact

SEQ ID NO: 80 - DNA, 10 bp, Artificial Sequence
  tag sequence for base balance
acttccgttc

SEQ ID NO: 81 - DNA, 10 bp, Artificial Sequence
  tag sequence for base balance
tgctccacga

SEQ ID NO: 82 - DNA, 10 bp, Artificial Sequence
  tag sequence for base balance
aatcaaggtc

SEQ ID NO: 83 - DNA, 10 bp, Artificial Sequence
  tag sequence for base balance
gtaggtcaat

SEQ ID NO: 84 - DNA, 10 bp, Artificial Sequence
  tag sequence for base balance
ccgatgttcg

SEQ ID NO: 85 - DNA, 10 bp, Artificial Sequence
  tag sequence for base balance
gacgtgtgca

SEQ ID NO: 86 - DNA, 10 bp, Artificial Sequence
  tag sequence for base balance
tcgccacttc

SEQ ID NO: 87 - DNA, 10 bp, Artificial Sequence
  tag sequence for base balance
ataagcacgt

SEQ ID NO: 88 - DNA, 10 bp, Artificial Sequence
  tag sequence for base balance
cgttatgaag

SEQ ID NO: 89 - DNA, 10 bp, Artificial Sequence
  tag sequence for base balance
aatagagcca

SEQ ID NO: 90 - DNA, 10 bp, Artificial Sequence
  tag sequence for base balance
gtacctcgac

SEQ ID NO: 91 - DNA, 10 bp, Artificial Sequence
  tag sequence for base balance
ccggtgattg

SEQ ID NO: 92 - DNA, 10 bp, Artificial Sequence
  tag sequence for base balance
tgctactagt

SEQ ID NO: 93 - DNA, 10 bp, Artificial Sequence
  tag sequence for base balance
gatccggact

SEQ ID NO: 94 - DNA, 10 bp, Artificial Sequence
  tag sequence for base balance
ttaggcacaa

SEQ ID NO: 95 - DNA, 10 bp, Artificial Sequence
  tag sequence for base balance
agcattcttg

SEQ ID NO: 96 - DNA, 10 bp, Artificial Sequence
  tag sequence for base balance
ccgtaatggc

SEQ ID NO: 97 - DNA, 10 bp, Artificial Sequence
  tag sequence for base balance
gtatagctgc

SEQ ID NO: 98 - DNA, 10 bp, Artificial Sequence
  tag sequence for base balance
cagacatctg

SEQ ID NO: 99 - DNA, 10 bp, Artificial Sequence
  tag sequence for base balance
agcggtggat

SEQ ID NO: 100 - DNA, 10 bp, Artificial Sequence
  tag sequence for base balance
tctctcaaca

SEQ ID NO: 101 - DNA, 10 bp, Artificial Sequence
  tag sequence for base balance
catccactgt

SEQ ID NO: 102 - DNA, 10 bp, Artificial Sequence
  tag sequence for base balance
gccgtgaaca

SEQ ID NO: 103 - DNA, 10 bp, Artificial Sequence
  tag sequence for base balance
ataagcggag

SEQ ID NO: 104 - DNA, 10 bp, Artificial Sequence
  tag sequence for base balance
tggtattctc

SEQ ID NO: 105 - DNA, 10 bp, Artificial Sequence
  tag sequence for base balance
acagttctca

SEQ ID NO: 106 - DNA, 10 bp, Artificial Sequence
  tag sequence for base balance
cattgagagc

SEQ ID NO: 107 - DNA, 10 bp, Artificial Sequence
  tag sequence for base balance
gtcacgactg

SEQ ID NO: 108 - DNA, 10 bp, Artificial Sequence
  tag sequence for base balance
tggcactgat

SEQ ID NO: 109 - DNA, 10 bp, Artificial Sequence
  tag sequence for base balance
aatgattcgc

SEQ ID NO: 110 - DNA, 10 bp, Artificial Sequence
  tag sequence for base balance
cgcttaagta

SEQ ID NO: 111 - DNA, 10 bp, Artificial Sequence
  tag sequence for base balance
ttgagcgacg

SEQ ID NO: 112 - DNA, 10 bp, Artificial Sequence
  tag sequence for base balance
gcaccgctat

SEQ ID NO: 113 - DNA, 10 bp, Artificial Sequence
  tag sequence for base balance
acgaacggat

SEQ ID NO: 114 - DNA, 10 bp, Artificial Sequence
  tag sequence for base balance
gaacggacta

SEQ ID NO: 115 - DNA, 10 bp, Artificial Sequence
  tag sequence for base balance
tgctctctgg

SEQ ID NO: 116 - DNA, 10 bp, Artificial Sequence
  tag sequence for base balance
cttgtatacc

SEQ ID NO: 117 - DNA, 10 bp, Artificial Sequence
  tag sequence for base balance
caccagcaca

SEQ ID NO: 118 - DNA, 10 bp, Artificial Sequence
  tag sequence for base balance
ttgtctgtag

SEQ ID NO: 119 - DNA, 10 bp, Artificial Sequence
  tag sequence for base balance
agtatcactc

SEQ ID NO: 120 - DNA, 10 bp, Artificial Sequence
  tag sequence for base balance
gcaggatggt

SEQ ID NO: 121 - DNA, 10 bp, Artificial Sequence
  tag sequence for base balance
ttatccacgt

SEQ ID NO: 122 - DNA, 10 bp, Artificial Sequence
  tag sequence for base balance
acggttcgtc

SEQ ID NO: 123 - DNA, 10 bp, Artificial Sequence
  tag sequence for base balance
gaccagtaag

SEQ ID NO: 124 - DNA, 10 bp, Artificial Sequence
  tag sequence for base balance
cgtagagtca

SEQ ID NO: 125 - DNA, 10 bp, Artificial Sequence
  tag sequence for base balance
acgttaaggt

SEQ ID NO: 126 - DNA, 10 bp, Artificial Sequence
  tag sequence for base balance
ctcagcttag

SEQ ID NO: 127 - DNA, 10 bp, Artificial Sequence
  tag sequence for base balance
tgtgctccta

SEQ ID NO: 128 - DNA, 10 bp, Artificial Sequence
  tag sequence for base balance
gaacaggacc

SEQ ID NO: 129 - DNA, 10 bp, Artificial Sequence
  tag sequence for base balance
gcgaccttga

SEQ ID NO: 130 - DNA, 10 bp, Artificial Sequence
  tag sequence for base balance
atcgtgagtt

SEQ ID NO: 131 - DNA, 10 bp, Artificial Sequence
  tag sequence for base balance
cgtcgtcaac

SEQ ID NO: 132 - DNA, 10 bp, Artificial Sequence
  tag sequence for base balance
taataagccg

SEQ ID NO: 133 - DNA, 10 bp, Artificial Sequence
  tag sequence for base balance
ccacttagta

SEQ ID NO: 134 - DNA, 10 bp, Artificial Sequence
  tag sequence for base balance
agtagctagt

SEQ ID NO: 135 - DNA, 10 bp, Artificial Sequence
  tag sequence for base balance
gacgaactcg

SEQ ID NO: 136 - DNA, 10 bp, Artificial Sequence
  tag sequence for base balance
ttgtcggcac

SEQ ID NO: 137 - DNA, 10 bp, Artificial Sequence
  tag sequence for base balance
agcatatcgt

SEQ ID NO: 138 - DNA, 10 bp, Artificial Sequence
  tag sequence for base balance
gtagacggag

SEQ ID NO: 139 - DNA, 10 bp, Artificial Sequence
  tag sequence for base balance
cattctcatc

SEQ ID NO: 140 - DNA, 10 bp, Artificial Sequence
  tag sequence for base balance
tcgcggatca

SEQ ID NO: 141 - DNA, 10 bp, Artificial Sequence
  tag sequence for base balance
ctggaggcaa

SEQ ID NO: 142 - DNA, 10 bp, Artificial Sequence
  tag sequence for base balance
gatacttgtg

SEQ ID NO: 143 - DNA, 10 bp, Artificial Sequence
  tag sequence for base balance
tgcctccact

SEQ ID NO: 144 - DNA, 10 bp, Artificial Sequence
  tag sequence for base balance
acatgaatgc

SEQ ID NO: 145 - DNA, 10 bp, Artificial Sequence
  tag sequence for base balance
tcagcagagg

SEQ ID NO: 146 - DNA, 10 bp, Artificial Sequence
  tag sequence for base balance
ctgtgcatta

SEQ ID NO: 147 - DNA, 10 bp, Artificial Sequence
  tag sequence for base balance
agtaatcgac

SEQ ID NO: 148 - DNA, 10 bp, Artificial Sequence
  tag sequence for base balance
agtaatcgac

SEQ ID NO: 149 - DNA, 10 bp, Artificial Sequence
  tag sequence for base balance
aagcggtgaa

SEQ ID NO: 150 - DNA, 10 bp, Artificial Sequence
  tag sequence for base balance
ctatcacact

SEQ ID NO: 151 - DNA, 10 bp, Artificial Sequence
  tag sequence for base balance
gccgttatgc

SEQ ID NO: 152 - DNA, 10 bp, Artificial Sequence
  tag sequence for base balance
tgtaacgctg

SEQ ID NO: 153 - DNA, 10 bp, Artificial Sequence
  tag sequence for base balance
gcgtgtaact

SEQ ID NO: 154 - DNA, 10 bp, Artificial Sequence
  tag sequence for base balance
catgtaccac

SEQ ID NO: 155 - DNA, 10 bp, Artificial Sequence
  tag sequence for base balance
tgccactgta

SEQ ID NO: 156 - DNA, 10 bp, Artificial Sequence
  tag sequence for base balance
ataacggtgg

SEQ ID NO: 157 - DNA, 10 bp, Artificial Sequence
  tag sequence for base balance
cttgaaggtt

SEQ ID NO: 158 - DNA, 10 bp, Artificial Sequence
  tag sequence for base balance
gcctctatgg

SEQ ID NO: 159 - DNA, 10 bp, Artificial Sequence
  tag sequence for base balance
tagatccacc

SEQ ID NO: 160 - DNA, 10 bp, Artificial Sequence
  tag sequence for base balance
agacggtcaa

SEQ ID NO: 161 - DNA, 10 bp, Artificial Sequence
  tag sequence for base balance
gctggattaa

SEQ ID NO: 162 - DNA, 10 bp, Artificial Sequence
  tag sequence for base balance
taacaccggc

SEQ ID NO: 163 - DNA, 10 bp, Artificial Sequence
  tag sequence for base balance
atgactgccg

SEQ ID NO: 164 - DNA, 10 bp, Artificial Sequence
  tag sequence for base balance
cgcttgaatt

SEQ ID NO: 165 - DNA, 10 bp, Artificial Sequence
  tag sequence for base balance
ctatagcgag

SEQ ID NO: 166 - DNA, 10 bp, Artificial Sequence
  tag sequence for base balance
aacgttgttc

SEQ ID NO: 167 - DNA, 10 bp, Artificial Sequence
  tag sequence for base balance
gctaccacgt

SEQ ID NO: 168 - DNA, 10 bp, Artificial Sequence
  tag sequence for base balance
tggcgataca

SEQ ID NO: 169 - DNA, 10 bp, Artificial Sequence
  tag sequence for base balance
tccgccaatc

SEQ ID NO: 170 - DNA, 10 bp, Artificial Sequence
  tag sequence for base balance
caactagtgt

SEQ ID NO: 171 - DNA, 10 bp, Artificial Sequence
  tag sequence for base balance
agtaagccaa

SEQ ID NO: 172 - DNA, 10 bp, Artificial Sequence
  tag sequence for base balance
gtgtgttgcg

SEQ ID NO: 173 - DNA, 10 bp, Artificial Sequence
  tag sequence for base balance
gatcagatgg

SEQ ID NO: 174 - DNA, 10 bp, Artificial Sequence
  tag sequence for base balance
ctcgtaggtc

SEQ ID NO: 175 - DNA, 10 bp, Artificial Sequence
  tag sequence for base balance
tcgtgtccat

SEQ ID NO: 176 - DNA, 10 bp, Artificial Sequence
  tag sequence for base balance
agaacctaca

SEQ ID NO: 177 - DNA, 10 bp, Artificial Sequence
  tag sequence for base balance
ccgcattcct

SEQ ID NO: 178 - DNA, 10 bp, Artificial Sequence
  tag sequence for base balance
gttggacata

SEQ ID NO: 179 - DNA, 10 bp, Artificial Sequence
  tag sequence for base balance
tgatcgaggc

SEQ ID NO: 180 - DNA, 10 bp, Artificial Sequence
  tag sequence for base balance
aacatcgtag

SEQ ID NO: 181 - DNA, 10 bp, Artificial Sequence
  tag sequence for base balance
gttgcgcgaa

SEQ ID NO: 182 - DNA, 10 bp, Artificial Sequence
  tag sequence for base balance
acaagtaagc

SEQ ID NO: 183 - DNA, 10 bp, Artificial Sequence
  tag sequence for base balance
cgcttctcct

SEQ ID NO: 184 - DNA, 10 bp, Artificial Sequence
  tag sequence for base balance
tagcaagttg

SEQ ID NO: 185 - DNA, 10 bp, Artificial Sequence
  tag sequence for base balance
aggcctcttc

SEQ ID NO: 186 - DNA, 10 bp, Artificial Sequence
  tag sequence for base balance
gtaatgtcgt

SEQ ID NO: 187 - DNA, 10 bp, Artificial Sequence
  tag sequence for base balance
cactgcagag

SEQ ID NO: 188 - DNA, 10 bp, Artificial Sequence
  tag sequence for base balance
tctgaagaca

SEQ ID NO: 189 - DNA, 10 bp, Artificial Sequence
  tag sequence for base balance
gctaaggata

SEQ ID NO: 190 - DNA, 10 bp, Artificial Sequence
  tag sequence for base balance
cacggttggt

SEQ ID NO: 191 - DNA, 10 bp, Artificial Sequence
  tag sequence for base balance
tgaccaccag

SEQ ID NO: 192 - DNA, 10 bp, Artificial Sequence
  tag sequence for base balance
atgttcatcc

SEQ ID NO: 193 - DNA, 10 bp, Artificial Sequence
  tag sequence for base balance
agctactctg

SEQ ID NO: 194 - DNA, 10 bp, Artificial Sequence
  tag sequence for base balance
caacgtgagt

SEQ ID NO: 195 - DNA, 10 bp, Artificial Sequence
  tag sequence for base balance
tcgatgctaa

SEQ ID NO: 196 - DNA, 10 bp, Artificial Sequence
  tag sequence for base balance
gttgcaagcc

SEQ ID NO: 197 - DNA, 10 bp, Artificial Sequence
  tag sequence for base balance
cgacatgtgt

SEQ ID NO: 198 - DNA, 10 bp, Artificial Sequence
  tag sequence for base balance
gatgcgcata

SEQ ID NO: 199 - DNA, 10 bp, Artificial Sequence
  tag sequence for base balance
tcgtgatcag

SEQ ID NO: 200 - DNA, 10 bp, Artificial Sequence
  tag sequence for base balance
atcatcagcc

SEQ ID NO: 201 - DNA, 10 bp, Artificial Sequence
  tag sequence for base balance
tcaatggcgg

SEQ ID NO: 202 - DNA, 10 bp, Artificial Sequence
  tag sequence for base balance
cagtaactct

SEQ ID NO: 203 - DNA, 10 bp, Artificial Sequence
  tag sequence for base balance
gttgcctgac

SEQ ID NO: 204 - DNA, 10 bp, Artificial Sequence
  tag sequence for base balance
agccgtaata

SEQ ID NO: 205 - DNA, 10 bp, Artificial Sequence
  tag sequence for base balance
ctaataggct

SEQ ID NO: 206 - DNA, 10 bp, Artificial Sequence
  tag sequence for base balance
tctcctccac

SEQ ID NO: 207 - DNA, 10 bp, Artificial Sequence
  tag sequence for base balance
agctgcatga

SEQ ID NO: 208 - DNA, 10 bp, Artificial Sequence
  tag sequence for base balance
gaggagtatg

SEQ ID NO: 209 - DNA, 10 bp, Artificial Sequence
  tag sequence for base balance
accacgtagc

SEQ ID NO: 210 - DNA, 10 bp, Artificial Sequence
  tag sequence for base balance
gaatgcagta

SEQ ID NO: 211 - DNA, 10 bp, Artificial Sequence
  tag sequence for base balance
ttggtagcct

SEQ ID NO: 212 - DNA, 10 bp, Artificial Sequence
  tag sequence for base balance
cgtcatctag

SEQ ID NO: 213 - DNA, 10 bp, Artificial Sequence
  tag sequence for base balance
tcaatgaggt

SEQ ID NO: 214 - DNA, 10 bp, Artificial Sequence
  tag sequence for base balance
agcgaagctg

SEQ ID NO: 215 - DNA, 10 bp, Artificial Sequence
  tag sequence for base balance
ctgtcttaac

SEQ ID NO: 216 - DNA, 10 bp, Artificial Sequence
  tag sequence for base balance
gatcgcctca

SEQ ID NO: 217 - DNA, 10 bp, Artificial Sequence
  tag sequence for base balance
gttccgaatg

SEQ ID NO: 218 - DNA, 10 bp, Artificial Sequence
  tag sequence for base balance
tacgtacgca

SEQ ID NO: 219 - DNA, 10 bp, Artificial Sequence
  tag sequence for base balance
cggagttcac

SEQ ID NO: 220 - DNA, 10 bp, Artificial Sequence
  tag sequence for base balance
acatacgtgt

SEQ ID NO: 221 - DNA, 10 bp, Artificial Sequence
  tag sequence for base balance
ctgaagagat

SEQ ID NO: 222 - DNA, 10 bp, Artificial Sequence
  tag sequence for base balance
gaagcctcca

SEQ ID NO: 223 - DNA, 10 bp, Artificial Sequence
  tag sequence for base balance
tgtcttcatc

SEQ ID NO: 224 - DNA, 10 bp, Artificial Sequence
  tag sequence for base balance
acctgagtgg

SEQ ID NO: 225 - DNA, 10 bp, Artificial Sequence
  tag sequence for base balance
gtacgtcctt

SEQ ID NO: 226 - DNA, 10 bp, Artificial Sequence
  tag sequence for base balance
aactaggtca

SEQ ID NO: 227 - DNA, 10 bp, Artificial Sequence
  tag sequence for base balance
tgtgtcaggc

SEQ ID NO: 228 - DNA, 10 bp, Artificial Sequence
  tag sequence for base balance
ccgacataag

SEQ ID NO: 229 - DNA, 10 bp, Artificial Sequence
  tag sequence for base balance
tccacacgtc

SEQ ID NO: 230 - DNA, 10 bp, Artificial Sequence
  tag sequence for base balance
cggcacatga

SEQ ID NO: 231 - DNA, 10 bp, Artificial Sequence
  tag sequence for base balance
gtatgttcct

SEQ ID NO: 232 - DNA, 10 bp, Artificial Sequence
  tag sequence for base balance
aatgtggaag

SEQ ID NO: 233 - DNA, 10 bp, Artificial Sequence
  tag sequence for base balance
agacagacgt

SEQ ID NO: 234 - DNA, 10 bp, Artificial Sequence
  tag sequence for base balance
ttctgtggag

SEQ ID NO: 235 - DNA, 10 bp, Artificial Sequence
  tag sequence for base balance
caggtcttcc

SEQ ID NO: 236 - DNA, 10 bp, Artificial Sequence
  tag sequence for base balance
gctacacata

SEQ ID NO: 237 - DNA, 10 bp, Artificial Sequence
  tag sequence for base balance
ctagcgacac

SEQ ID NO: 238 - DNA, 10 bp, Artificial Sequence
  tag sequence for base balance
aggcattact

SEQ ID NO: 239 - DNA, 10 bp, Artificial Sequence
  tag sequence for base balance
gacatccgga

SEQ ID NO: 240 - DNA, 10 bp, Artificial Sequence
  tag sequence for base balance
tcttgagttg

SEQ ID NO: 241 - DNA, 10 bp, Artificial Sequence
  tag sequence for base balance
acaacagaag

SEQ ID NO: 242 - DNA, 10 bp, Artificial Sequence
  tag sequence for base balance
cgcttgtgga

SEQ ID NO: 243 - DNA, 10 bp, Artificial Sequence
  tag sequence for base balance
gttggtctcc

SEQ ID NO: 244 - DNA, 10 bp, Artificial Sequence
  tag sequence for base balance
tagcacactt

SEQ ID NO: 245 - DNA, 10 bp, Artificial Sequence
  tag sequence for base balance
gcttgcaata

SEQ ID NO: 246 - DNA, 10 bp, Artificial Sequence
  tag sequence for base balance
tggacgtgct

SEQ ID NO: 247 - DNA, 10 bp, Artificial Sequence
  tag sequence for base balance
aacgaaccgg

SEQ ID NO: 248 - DNA, 10 bp, Artificial Sequence
  tag sequence for base balance
ctacttgtac

SEQ ID NO: 249 - DNA, 10 bp, Artificial Sequence
  tag sequence for base balance
cggtgagtga

SEQ ID NO: 250 - DNA, 10 bp, Artificial Sequence
  tag sequence for base balance
gcaatgcatt

SEQ ID NO: 251 - DNA, 10 bp, Artificial Sequence
  tag sequence for base balance
ttccattcac

SEQ ID NO: 252 - DNA, 10 bp, Artificial Sequence
  tag sequence for base balance
aatgccagcg

SEQ ID NO: 253 - DNA, 10 bp, Artificial Sequence
  tag sequence for base balance
tactcttctc

SEQ ID NO: 254 - DNA, 10 bp, Artificial Sequence
  tag sequence for base balance
aggaaggtaa

SEQ ID NO: 255 - DNA, 10 bp, Artificial Sequence
  tag sequence for base balance
gttggacggt

SEQ ID NO: 256 - DNA, 10 bp, Artificial Sequence
  tag sequence for base balance
ccactcaacg

SEQ ID NO: 257 - DNA, 10 bp, Artificial Sequence
  tag sequence for base balance
aatgactggt

SEQ ID NO: 258 - DNA, 10 bp, Artificial Sequence
  tag sequence for base balance
gtgccacaac

SEQ ID NO: 259 - DNA, 10 bp, Artificial Sequence
  tag sequence for base balance
cgaatgatcg

SEQ ID NO: 260 - DNA, 10 bp, Artificial Sequence
  tag sequence for base balance
tcctgtgcta

SEQ ID NO: 261 - DNA, 10 bp, Artificial Sequence
  tag sequence for base balance
tgtgaattgg

SEQ ID NO: 262 - DNA, 10 bp, Artificial Sequence
  tag sequence for base balance
aaccggcctt

SEQ ID NO: 263 - DNA, 10 bp, Artificial Sequence
  tag sequence for base balance
ctatccgacc

SEQ ID NO: 264 - DNA, 10 bp, Artificial Sequence
  tag sequence for base balance
gcgattagaa

SEQ ID NO: 265 - DNA, 10 bp, Artificial Sequence
  tag sequence for base balance
cgtaaccgca

SEQ ID NO: 266 - DNA, 10 bp, Artificial Sequence
  tag sequence for base balance
gactgataac

SEQ ID NO: 267 - DNA, 10 bp, Artificial Sequence
  tag sequence for base balance
atgcttactg

SEQ ID NO: 268 - DNA, 10 bp, Artificial Sequence
  tag sequence for base balance
tcagcggtgt

SEQ ID NO: 269 - DNA, 10 bp, Artificial Sequence
  tag sequence for base balance
acataacacc

SEQ ID NO: 270 - DNA, 10 bp, Artificial Sequence
  tag sequence for base balance
cacctgaggt

SEQ ID NO: 271 - DNA, 10 bp, Artificial Sequence
  tag sequence for base balance
gtgactgtaa

SEQ ID NO: 272 - DNA, 10 bp, Artificial Sequence
  tag sequence for base balance
tgtggctctg

SEQ ID NO: 273 - DNA, 10 bp, Artificial Sequence
  tag sequence for base balance
ctcagactct

SEQ ID NO: 274 - DNA, 10 bp, Artificial Sequence
  tag sequence for base balance
acacatgcta

SEQ ID NO: 275 - DNA, 10 bp, Artificial Sequence
  tag sequence for base balance
tgtgcctaag

SEQ ID NO: 276 - DNA, 10 bp, Artificial Sequence
  tag sequence for base balance
gagttgaggc

SEQ ID NO: 277 - DNA, 10 bp, Artificial Sequence
  tag sequence for base balance
agccgttctc

SEQ ID NO: 278 - DNA, 10 bp, Artificial Sequence
  tag sequence for base balance
ttgttggtct

SEQ ID NO: 279 - DNA, 10 bp, Artificial Sequence
  tag sequence for base balance
caagacaaga

SEQ ID NO: 280 - DNA, 10 bp, Artificial Sequence
  tag sequence for base balance
gctacacgag

SEQ ID NO: 281 - DNA, 10 bp, Artificial Sequence
  tag sequence for base balance
gtgacgcgat

SEQ ID NO: 282 - DNA, 10 bp, Artificial Sequence
  tag sequence for base balance
aacctctctg

SEQ ID NO: 283 - DNA, 10 bp, Artificial Sequence
  tag sequence for base balance
tcttgagaga

SEQ ID NO: 284 - DNA, 10 bp, Artificial Sequence
  tag sequence for base balance
cgagatatcc

SEQ ID NO: 285 - DNA, 10 bp, Artificial Sequence
  tag sequence for base balance
gaaggattca

SEQ ID NO: 286 - DNA, 10 bp, Artificial Sequence
  tag sequence for base balance
tcgcctggtt

SEQ ID NO: 287 - DNA, 10 bp, Artificial Sequence
  tag sequence for base balance
agtaacacgg

SEQ ID NO: 288 - DNA, 10 bp, Artificial Sequence
  tag sequence for base balance
ctcttgcaac

SEQ ID NO: 289 - DNA, 10 bp, Artificial Sequence
  tag sequence for base balance
agagacttac

SEQ ID NO: 290 - DNA, 10 bp, Artificial Sequence
  tag sequence for base balance
cttatggccg

SEQ ID NO: 291 - DNA, 10 bp, Artificial Sequence
  tag sequence for base balance
gcctgacgtt

SEQ ID NO: 292 - DNA, 10 bp, Artificial Sequence
  tag sequence for base balance
tagcctaaga

SEQ ID NO: 293 - DNA, 10 bp, Artificial Sequence
  tag sequence for base balance
aagcatatcc

SEQ ID NO: 294 - DNA, 10 bp, Artificial Sequence
  tag sequence for base balance
ctaatccgtt

SEQ ID NO: 295 - DNA, 10 bp, Artificial Sequence
  tag sequence for base balance
gcttggtcga

SEQ ID NO: 296 - DNA, 10 bp, Artificial Sequence
  tag sequence for base balance
tgcgcagaag

SEQ ID NO: 297 - DNA, 10 bp, Artificial Sequence
  tag sequence for base balance
gatcctgata

SEQ ID NO: 298 - DNA, 10 bp, Artificial Sequence
  tag sequence for base balance
tcaagcacgg

SEQ ID NO: 299 - DNA, 10 bp, Artificial Sequence
  tag sequence for base balance
ctgtagcgct

SEQ ID NO: 300 - DNA, 10 bp, Artificial Sequence
  tag sequence for base balance
agcgtattac

SEQ ID NO: 301 - DNA, 10 bp, Artificial Sequence
  tag sequence for base balance
tgtctgattg

SEQ ID NO: 302 - DNA, 10 bp, Artificial Sequence
  tag sequence for base balance
accagacggt

SEQ ID NO: 303 - DNA, 10 bp, Artificial Sequence
  tag sequence for base balance
gtgtctgacc

SEQ ID NO: 304 - DNA, 10 bp, Artificial Sequence
  tag sequence for base balance
caagactcaa

SEQ ID NO: 305 - DNA, 10 bp, Artificial Sequence
  tag sequence for base balance
caagactcaa

SEQ ID NO: 306 - DNA, 10 bp, Artificial Sequence
  tag sequence for base balance
agacgaggtc

SEQ ID NO: 307 - DNA, 10 bp, Artificial Sequence
  tag sequence for base balance
ctggattact

SEQ ID NO: 308 - DNA, 10 bp, Artificial Sequence
  tag sequence for base balance
gatatgctga

SEQ ID NO: 309 - DNA, 10 bp, Artificial Sequence
  tag sequence for base balance
ctggtcaagg

SEQ ID NO: 310 - DNA, 10 bp, Artificial Sequence
  tag sequence for base balance
gctccattcc

SEQ ID NO: 311 - DNA, 10 bp, Artificial Sequence
  tag sequence for base balance
tgatgtcgaa

SEQ ID NO: 312 - DNA, 10 bp, Artificial Sequence
  tag sequence for base balance
aacaaggctt

SEQ ID NO: 313 - DNA, 10 bp, Artificial Sequence
  tag sequence for base balance
catctagaca

SEQ ID NO: 314 - DNA, 10 bp, Artificial Sequence
  tag sequence for base balance
gcggatacag

SEQ ID NO: 315 - DNA, 10 bp, Artificial Sequence
  tag sequence for base balance
ttctgcttgt

SEQ ID NO: 316 - DNA, 10 bp, Artificial Sequence
  tag sequence for base balance
agaacgcgtc

SEQ ID NO: 317 - DNA, 10 bp, Artificial Sequence
  tag sequence for base balance
aagacgaact

SEQ ID NO: 318 - DNA, 10 bp, Artificial Sequence
  tag sequence for base balance
ccagtactgc

SEQ ID NO: 319 - DNA, 10 bp, Artificial Sequence
  tag sequence for base balance
gttcgctgta

SEQ ID NO: 320 - DNA, 10 bp, Artificial Sequence
  tag sequence for base balance
tgctatgcag

SEQ ID NO: 321 - DNA, 10 bp, Artificial Sequence
  tag sequence for base balance
tacacgcgca

SEQ ID NO: 322 - DNA, 10 bp, Artificial Sequence
  tag sequence for base balance
aggtacgcag

SEQ ID NO: 323 - DNA, 10 bp, Artificial Sequence
  tag sequence for base balance
gttcgattgt

SEQ ID NO: 324 - DNA, 10 bp, Artificial Sequence
  tag sequence for base balance
ccagttaatc

SEQ ID NO: 325 - DNA, 10 bp, Artificial Sequence
  tag sequence for base balance
taagatcgga

SEQ ID NO: 326 - DNA, 10 bp, Artificial Sequence
  tag sequence for base balance
agctcggctt

SEQ ID NO: 327 - DNA, 10 bp, Artificial Sequence
  tag sequence for base balance
gttcgataag

SEQ ID NO: 328 - DNA, 10 bp, Artificial Sequence
  tag sequence for base balance
ccgatcatcc

SEQ ID NO: 329 - DNA, 10 bp, Artificial Sequence
  tag sequence for base balance
actggactca

SEQ ID NO: 330 - DNA, 10 bp, Artificial Sequence
  tag sequence for base balance
caatagaggc

SEQ ID NO: 331 - DNA, 10 bp, Artificial Sequence
  tag sequence for base balance
gtcacttaag

SEQ ID NO: 332 - DNA, 10 bp, Artificial Sequence
  tag sequence for base balance
tggctcgctt

SEQ ID NO: 333 - DNA, 10 bp, Artificial Sequence
  tag sequence for base balance
cgcactatgg

SEQ ID NO: 334 - DNA, 10 bp, Artificial Sequence
  tag sequence for base balance
gaggtacatt

SEQ ID NO: 335 - DNA, 10 bp, Artificial Sequence
  tag sequence for base balance
tcttagtgac

SEQ ID NO: 336 - DNA, 10 bp, Artificial Sequence
  tag sequence for base balance
atacgcgcca

SEQ ID NO: 337 - DNA, 10 bp, Artificial Sequence
  tag sequence for base balance
tgaggcatat

SEQ ID NO: 338 - DNA, 10 bp, Artificial Sequence
  tag sequence for base balance
attctatggc

SEQ ID NO: 339 - DNA, 10 bp, Artificial Sequence
  tag sequence for base balance
ccgtagcatg

SEQ ID NO: 340 - DNA, 10 bp, Artificial Sequence
  tag sequence for base balance
gacactgcca

SEQ ID NO: 341 - DNA, 10 bp, Artificial Sequence
  tag sequence for base balance
acggcattaa

SEQ ID NO: 342 - DNA, 10 bp, Artificial Sequence
  tag sequence for base balance
gtaagcgagg

SEQ ID NO: 343 - DNA, 10 bp, Artificial Sequence
  tag sequence for base balance
cattatcgct

SEQ ID NO: 344 - DNA, 10 bp, Artificial Sequence
  tag sequence for base balance
tgcctgactc

SEQ ID NO: 345 - DNA, 10 bp, Artificial Sequence
  tag sequence for base balance
gactcatcca

SEQ ID NO: 346 - DNA, 10 bp, Artificial Sequence
  tag sequence for base balance
acgaacatac

SEQ ID NO: 347 - DNA, 10 bp, Artificial Sequence
  tag sequence for base balance
ttacgtcggt

SEQ ID NO: 348 - DNA, 10 bp, Artificial Sequence
  tag sequence for base balance
cgtgtggatg

SEQ ID NO: 349 - DNA, 10 bp, Artificial Sequence
  tag sequence for base balance
cctaacattc

SEQ ID NO: 350 - DNA, 10 bp, Artificial Sequence
  tag sequence for base balance
atcgcacgca

SEQ ID NO: 351 - DNA, 10 bp, Artificial Sequence
  tag sequence for base balance
gaacgttcgg

SEQ ID NO: 352 - DNA, 10 bp, Artificial Sequence
  tag sequence for base balance
tggttggaat

SEQ ID NO: 353 - DNA, 10 bp, Artificial Sequence
  tag sequence for base balance
aacaagtgag

SEQ ID NO: 354 - DNA, 10 bp, Artificial Sequence
  tag sequence for base balance
gttgttgctc

SEQ ID NO: 355 - DNA, 10 bp, Artificial Sequence
  tag sequence for base balance
tgacgcaact

SEQ ID NO: 356 - DNA, 10 bp, Artificial Sequence
  tag sequence for base balance
ccgtcactga

SEQ ID NO: 357 - DNA, 10 bp, Artificial Sequence
  tag sequence for base balance
tgttattccg

SEQ ID NO: 358 - DNA, 10 bp, Artificial Sequence
  tag sequence for base balance
ctactcaaga

SEQ ID NO: 359 - DNA, 10 bp, Artificial Sequence
  tag sequence for base balance
acgagacgtc

SEQ ID NO: 360 - DNA, 10 bp, Artificial Sequence
  tag sequence for base balance
gacgcggtat

SEQ ID NO: 361 - DNA, 10 bp, Artificial Sequence
  tag sequence for base balance
gatgacgtta

SEQ ID NO: 362 - DNA, 10 bp, Artificial Sequence
  tag sequence for base balance
agccgatacc

SEQ ID NO: 363 - DNA, 10 bp, Artificial Sequence
  tag sequence for base balance
ttatctcgag

SEQ ID NO: 364 - DNA, 10 bp, Artificial Sequence
  tag sequence for base balance
ccgatgacgt

SEQ ID NO: 365 - DNA, 10 bp, Artificial Sequence
  tag sequence for base balance
gtgagttcgc

SEQ ID NO: 366 - DNA, 10 bp, Artificial Sequence
  tag sequence for base balance
acacaacatg

SEQ ID NO: 367 - DNA, 10 bp, Artificial Sequence
  tag sequence for base balance
cgtgcgatca

SEQ ID NO: 368 - DNA, 10 bp, Artificial Sequence
  tag sequence for base balance
tacttcggat

SEQ ID NO: 369 - DNA, 10 bp, Artificial Sequence
  tag sequence for base balance
ctatcggtgt

SEQ ID NO: 370 - DNA, 10 bp, Artificial Sequence
  tag sequence for base balance
gacattcaag

SEQ ID NO: 371 - DNA, 10 bp, Artificial Sequence
  tag sequence for base balance
agtgacacca

SEQ ID NO: 372 - DNA, 10 bp, Artificial Sequence
  tag sequence for base balance
tcgcgatgtc

SEQ ID NO: 373 - DNA, 10 bp, Artificial Sequence
  tag sequence for base balance
cgagtcagtc

SEQ ID NO: 374 - DNA, 10 bp, Artificial Sequence
  tag sequence for base balance
ttgccagtga

SEQ ID NO: 375 - DNA, 10 bp, Artificial Sequence
  tag sequence for base balance
aacaagcact

SEQ ID NO: 376 - DNA, 10 bp, Artificial Sequence
  tag sequence for base balance
gcttgttcag

SEQ ID NO: 377 - DNA, 10 bp, Artificial Sequence
  tag sequence for base balance
tagtgatgtg

SEQ ID NO: 378 - DNA, 10 bp, Artificial Sequence
  tag sequence for base balance
cgtgtgacat

SEQ ID NO: 379 - DNA, 10 bp, Artificial Sequence
  tag sequence for base balance
atccaccacc

SEQ ID NO: 380 - DNA, 10 bp, Artificial Sequence
  tag sequence for base balance
gcaactgtga

SEQ ID NO: 381 - DNA, 10 bp, Artificial Sequence
  tag sequence for base balance
atccaccggt

SEQ ID NO: 382 - DNA, 10 bp, Artificial Sequence
  tag sequence for base balance
ccgtcattac

SEQ ID NO: 383 - DNA, 10 bp, Artificial Sequence
  tag sequence for base balance
tgagtggcta

SEQ ID NO: 384 - DNA, 10 bp, Artificial Sequence
  tag sequence for base balance
gatagtaacg

SEQ ID NO: 385 - DNA, 10 bp, Artificial Sequence
  tag sequence for base balance
cgtcgatgac

SEQ ID NO: 386 - DNA, 10 bp, Artificial Sequence
  tag sequence for base balance
atataaggcg

SEQ ID NO: 387 - DNA, 10 bp, Artificial Sequence
  tag sequence for base balance
gatcgtgctc

SEQ ID NO: 388 - DNA, 10 bp, Artificial Sequence
  tag sequence for base balance
cagtcttcgg

SEQ ID NO: 389 - DNA, 10 bp, Artificial Sequence
  tag sequence for base balance
agaacgatct

SEQ ID NO: 390 - DNA, 10 bp, Artificial Sequence
  tag sequence for base balance
ttggtgcatt

SEQ ID NO: 391 - DNA, 10 bp, Artificial Sequence
  tag sequence for base balance
gccgtcataa

SEQ ID NO: 392 - DNA, 10 bp, Artificial Sequence
  tag sequence for base balance
tccaaccaga

SEQ ID NO: 393 - DNA, 10 bp, Artificial Sequence
  tag sequence for base balance
gatagcaaga

SEQ ID NO: 394 - DNA, 10 bp, Artificial Sequence
  tag sequence for base balance
accgtgcttc

SEQ ID NO: 395 - DNA, 10 bp, Artificial Sequence
  tag sequence for base balance
gcagatgtaa

SEQ ID NO: 396 - DNA, 10 bp, Artificial Sequence
  tag sequence for base balance
tgttggagcg

SEQ ID NO: 397 - DNA, 10 bp, Artificial Sequence
  tag sequence for base balance
ttgtatccac

SEQ ID NO: 398 - DNA, 10 bp, Artificial Sequence
  tag sequence for base balance
cgcacagatg

SEQ ID NO: 399 - DNA, 10 bp, Artificial Sequence
  tag sequence for base balance
caactctcgt

SEQ ID NO: 400 - DNA, 10 bp, Artificial Sequence
  tag sequence for base balance
atgccatgct

SEQ ID NO: 401 - DNA, 10 bp, Artificial Sequence
  tag sequence for base balance
aggcagctta

SEQ ID NO: 402 - DNA, 10 bp, Artificial Sequence
  tag sequence for base balance
tagcctagcg

SEQ ID NO: 403 - DNA, 10 bp, Artificial Sequence
  tag sequence for base balance
atcacgtgcg

SEQ ID NO: 404 - DNA, 10 bp, Artificial Sequence
  tag sequence for base balance
cgttatgcgc

SEQ ID NO: 405 - DNA, 10 bp, Artificial Sequence
  tag sequence for base balance
caaggatcga

SEQ ID NO: 406 - DNA, 10 bp, Artificial Sequence
  tag sequence for base balance
gttgtcgtat

SEQ ID NO: 407 - DNA, 10 bp, Artificial Sequence
  tag sequence for base balance
gcaatcaatc

SEQ ID NO: 408 - DNA, 10 bp, Artificial Sequence
  tag sequence for base balance
tcctgacaat

SEQ ID NO: 409 - DNA, 10 bp, Artificial Sequence
  tag sequence for base balance
aggtgcctta

SEQ ID NO: 410 - DNA, 10 bp, Artificial Sequence
  tag sequence for base balance
aagaaccaag

SEQ ID NO: 411 - DNA, 10 bp, Artificial Sequence
  tag sequence for base balance
catacatgac

SEQ ID NO: 412 - DNA, 10 bp, Artificial Sequence
  tag sequence for base balance
tgcctggtga

SEQ ID NO: 413 - DNA, 10 bp, Artificial Sequence
  tag sequence for base balance
tctcggagtt

SEQ ID NO: 414 - DNA, 10 bp, Artificial Sequence
  tag sequence for base balance
gtcgtagact

SEQ ID NO: 415 - DNA, 10 bp, Artificial Sequence
  tag sequence for base balance
gcatataccg

SEQ ID NO: 416 - DNA, 10 bp, Artificial Sequence
  tag sequence for base balance
ctagcttcgc

SEQ ID NO: 417 - DNA, 10 bp, Artificial Sequence
  tag sequence for base balance
gacgtatcaa

SEQ ID NO: 418 - DNA, 10 bp, Artificial Sequence
  tag sequence for base balance
cctgctagga

SEQ ID NO: 419 - DNA, 10 bp, Artificial Sequence
  tag sequence for base balance
caacttggcg

SEQ ID NO: 420 - DNA, 10 bp, Artificial Sequence
  tag sequence for base balance
atgcgacctc

SEQ ID NO: 421 - DNA, 10 bp, Artificial Sequence
  tag sequence for base balance
gttaaggacg

SEQ ID NO: 422 - DNA, 10 bp, Artificial Sequence
  tag sequence for base balance
tccaagttgt

SEQ ID NO: 423 - DNA, 10 bp, Artificial Sequence
  tag sequence for base balance
aggtccattc

SEQ ID NO: 424 - DNA, 10 bp, Artificial Sequence
  tag sequence for base balance
tgatgccaat

SEQ ID NO: 425 - DNA, 10 bp, Artificial Sequence
  tag sequence for base balance
cctaagagtt

SEQ ID NO: 426 - DNA, 10 bp, Artificial Sequence
  tag sequence for base balance
gatactagct

SEQ ID NO: 427 - DNA, 10 bp, Artificial Sequence
  tag sequence for base balance
aaggcatctc

SEQ ID NO: 428 - DNA, 10 bp, Artificial Sequence
  tag sequence for base balance
tggcatctgg

SEQ ID NO: 429 - DNA, 10 bp, Artificial Sequence
  tag sequence for base balance
acactggagc

SEQ ID NO: 430 - DNA, 10 bp, Artificial Sequence
  tag sequence for base balance
gtatgccaca

SEQ ID NO: 431 - DNA, 10 bp, Artificial Sequence
  tag sequence for base balance
ctcttagtag

SEQ ID NO: 432 - DNA, 10 bp, Artificial Sequence
  tag sequence for base balance
tgcggctcaa

SEQ ID NO: 433 - DNA, 10 bp, Artificial Sequence
  tag sequence for base balance
taaggctaga

SEQ ID NO: 434 - DNA, 10 bp, Artificial Sequence
  tag sequence for base balance
gaggagataa

SEQ ID NO: 435 - DNA, 10 bp, Artificial Sequence
  tag sequence for base balance
cgttagcact

SEQ ID NO: 436 - DNA, 10 bp, Artificial Sequence
  tag sequence for base balance
aggctaggat

SEQ ID NO: 437 - DNA, 10 bp, Artificial Sequence
  tag sequence for base balance
atctcactgg

SEQ ID NO: 438 - DNA, 10 bp, Artificial Sequence
  tag sequence for base balance
tccagttctc

SEQ ID NO: 439 - DNA, 10 bp, Artificial Sequence
  tag sequence for base balance
gtaaccgctc

SEQ ID NO: 440 - DNA, 10 bp, Artificial Sequence
  tag sequence for base balance
cctcttagcg

SEQ ID NO: 441 - DNA, 10 bp, Artificial Sequence
  tag sequence for base balance
actaaggctg

SEQ ID NO: 442 - DNA, 10 bp, Artificial Sequence
  tag sequence for base balance
gaggagtatg

SEQ ID NO: 443 - DNA, 10 bp, Artificial Sequence
  tag sequence for base balance
tagtcaacgc

SEQ ID NO: 444 - DNA, 10 bp, Artificial Sequence
  tag sequence for base balance
ccatcaagga

SEQ ID NO: 445 - DNA, 10 bp, Artificial Sequence
  tag sequence for base balance
agcctctgct

SEQ ID NO: 446 - DNA, 10 bp, Artificial Sequence
  tag sequence for base balance
ttcgttcaca

SEQ ID NO: 447 - DNA, 10 bp, Artificial Sequence
  tag sequence for base balance
gtaagtgtac

SEQ ID NO: 448 - DNA, 10 bp, Artificial Sequence
  tag sequence for base balance
cgtcgcctat

SEQ ID NO: 449 - DNA, 10 bp, Artificial Sequence
  tag sequence for base balance
tgtgaaggag

SEQ ID NO: 450 - DNA, 10 bp, Artificial Sequence
  tag sequence for base balance
agaccggttc

SEQ ID NO: 451 - DNA, 10 bp, Artificial Sequence
  tag sequence for base balance
ctcgcctaac

SEQ ID NO: 452 - DNA, 10 bp, Artificial Sequence
  tag sequence for base balance
ccgctgtcta

SEQ ID NO: 453 - DNA, 10 bp, Artificial Sequence
  tag sequence for base balance
gacataacct

SEQ ID NO: 454 - DNA, 10 bp, Artificial Sequence
  tag sequence for base balance
gagaatagca

SEQ ID NO: 455 - DNA, 10 bp, Artificial Sequence
  tag sequence for base balance
ttatgtcagg

SEQ ID NO: 456 - DNA, 10 bp, Artificial Sequence
  tag sequence for base balance
acttgcctgt

SEQ ID NO: 457 - DNA, 10 bp, Artificial Sequence
  tag sequence for base balance
tgctggatct

SEQ ID NO: 458 - DNA, 10 bp, Artificial Sequence
  tag sequence for base balance
agtagtgttg

SEQ ID NO: 459 - DNA, 10 bp, Artificial Sequence
  tag sequence for base balance
ctccaatcct

SEQ ID NO: 460 - DNA, 10 bp, Artificial Sequence
  tag sequence for base balance
cctatgtgta

SEQ ID NO: 461 - DNA, 10 bp, Artificial Sequence
  tag sequence for base balance
taatatccgc

SEQ ID NO: 462 - DNA, 10 bp, Artificial Sequence
  tag sequence for base balance
gtgccacaac

SEQ ID NO: 463 - DNA, 10 bp, Artificial Sequence
  tag sequence for base balance
gcagtcagga

SEQ ID NO: 464 - DNA, 10 bp, Artificial Sequence
  tag sequence for base balance
aaggccgaag

SEQ ID NO: 465 - DNA, 10 bp, Artificial Sequence
  tag sequence for base balance
cgtgttagag

SEQ ID NO: 466 - DNA, 10 bp, Artificial Sequence
  tag sequence for base balance
acaggacgat

SEQ ID NO: 467 - DNA, 10 bp, Artificial Sequence
  tag sequence for base balance
cggataacgg

SEQ ID NO: 468 - DNA, 10 bp, Artificial Sequence
  tag sequence for base balance
gttagtgcct

SEQ ID NO: 469 - DNA, 10 bp, Artificial Sequence
  tag sequence for base balance
aagcacgaca

SEQ ID NO: 470 - DNA, 10 bp, Artificial Sequence
  tag sequence for base balance
gtctccttgc

SEQ ID NO: 471 - DNA, 10 bp, Artificial Sequence
  tag sequence for base balance
tcaccgtata

SEQ ID NO: 472 - DNA, 10 bp, Artificial Sequence
  tag sequence for base balance
tactagcttc

SEQ ID NO: 473 - DNA, 10 bp, Artificial Sequence
  tag sequence for base balance
accattcacg

SEQ ID NO: 474 - DNA, 10 bp, Artificial Sequence
  tag sequence for base balance
agtagctagt

SEQ ID NO: 475 - DNA, 10 bp, Artificial Sequence
  tag sequence for base balance
ttccgaaggt

SEQ ID NO: 476 - DNA, 10 bp, Artificial Sequence
  tag sequence for base balance
gtaccaacca

SEQ ID NO: 477 - DNA, 10 bp, Artificial Sequence
  tag sequence for base balance
tatgtgtgtc

SEQ ID NO: 478 - DNA, 10 bp, Artificial Sequence
  tag sequence for base balance
cgatcggtac

SEQ ID NO: 479 - DNA, 10 bp, Artificial Sequence
  tag sequence for base balance
gaggatctag

SEQ ID NO: 480 - DNA, 10 bp, Artificial Sequence
  tag sequence for base balance
ccgtacgcta

SEQ ID NO: 481 - DNA, 10 bp, Artificial Sequence
  tag sequence for base balance
gtcaactcgg

SEQ ID NO: 482 - DNA, 10 bp, Artificial Sequence
  tag sequence for base balance
tggaagcaca

SEQ ID NO: 483 - DNA, 10 bp, Artificial Sequence
  tag sequence for base balance
tcgttgtagc

SEQ ID NO: 484 - DNA, 10 bp, Artificial Sequence
  tag sequence for base balance
agccgaagtt

SEQ ID NO: 485 - DNA, 10 bp, Artificial Sequence
  tag sequence for base balance
gatgcaacct

SEQ ID NO: 486 - DNA, 10 bp, Artificial Sequence
  tag sequence for base balance
acttccgttc

SEQ ID NO: 487 - DNA, 10 bp, Artificial Sequence
  tag sequence for base balance
caagttggaa

SEQ ID NO: 488 - DNA, 10 bp, Artificial Sequence
  tag sequence for base balance
ctacgtctag

SEQ ID NO: 489 - DNA, 10 bp, Artificial Sequence
  tag sequence for base balance
tgtcgttaag

SEQ ID NO: 490 - DNA, 10 bp, Artificial Sequence
  tag sequence for base balance
gtctcaatga

SEQ ID NO: 491 - DNA, 10 bp, Artificial Sequence
  tag sequence for base balance
gatcaagcca

SEQ ID NO: 492 - DNA, 10 bp, Artificial Sequence
  tag sequence for base balance
aactccgatc

SEQ ID NO: 493 - DNA, 10 bp, Artificial Sequence
  tag sequence for base balance
ctaagtcttc

SEQ ID NO: 494 - DNA, 10 bp, Artificial Sequence
  tag sequence for base balance
tgagagcgct

SEQ ID NO: 495 - DNA, 10 bp, Artificial Sequence
  tag sequence for base balance
acgatctcgg

SEQ ID NO: 496 - DNA, 10 bp, Artificial Sequence
  tag sequence for base balance
ccggtgagat

SEQ ID NO: 497 - DNA, 10 bp, Artificial Sequence
  tag sequence for base balance
catctcatga

SEQ ID NO: 498 - DNA, 10 bp, Artificial Sequence
  tag sequence for base balance
ctgtgactcg

SEQ ID NO: 499 - DNA, 10 bp, Artificial Sequence
  tag sequence for base balance
agaccttgga

SEQ ID NO: 500 - DNA, 10 bp, Artificial Sequence
  tag sequence for base balance
actgtcgacg

SEQ ID NO: 501 - DNA, 10 bp, Artificial Sequence
  tag sequence for base balance
gtgaagacac

SEQ ID NO: 502 - DNA, 10 bp, Artificial Sequence
  tag sequence for base balance
tactgtgcat

SEQ ID NO: 503 - DNA, 10 bp, Artificial Sequence
  tag sequence for base balance
gcagagcgtt

SEQ ID NO: 504 - DNA, 10 bp, Artificial Sequence
  tag sequence for base balance
tgcacatatc

SEQ ID NO: 505 - DNA, 10 bp, Artificial Sequence
  tag sequence for base balance
cctgtgtaac

SEQ ID NO: 506 - DNA, 10 bp, Artificial Sequence
  tag sequence for base balance
aacgatgcca

SEQ ID NO: 507 - DNA, 10 bp, Artificial Sequence
  tag sequence for base balance
tcgagcatag

SEQ ID NO: 508 - DNA, 10 bp, Artificial Sequence
  tag sequence for base balance
gaattcctgt

SEQ ID NO: 509 - DNA, 10 bp, Artificial Sequence
  tag sequence for base balance
agaacgtccg

SEQ ID NO: 510 - DNA, 10 bp, Artificial Sequence
  tag sequence for base balance
cgccaaggta

SEQ ID NO: 511 - DNA, 10 bp, Artificial Sequence
  tag sequence for base balance
ttgtgaaggc

SEQ ID NO: 512 - DNA, 10 bp, Artificial Sequence
  tag sequence for base balance
gttcctcatt

SEQ ID NO: 513 - DNA, 10 bp, Artificial Sequence
  tag sequence for base balance
cgtcactatt

SEQ ID NO: 514 - DNA, 10 bp, Artificial Sequence
  tag sequence for base balance
gcgatgcaga

SEQ ID NO: 515 - DNA, 10 bp, Artificial Sequence
  tag sequence for base balance
cgtgtcctag

SEQ ID NO: 516 - DNA, 10 bp, Artificial Sequence
  tag sequence for base balance
gaagaatgga

SEQ ID NO: 517 - DNA, 10 bp, Artificial Sequence
  tag sequence for base balance
atgtgtggct

SEQ ID NO: 518 - DNA, 10 bp, Artificial Sequence
  tag sequence for base balance
tcctgtacac

SEQ ID NO: 519 - DNA, 10 bp, Artificial Sequence
  tag sequence for base balance
ttaccgattc

SEQ ID NO: 520 - DNA, 10 bp, Artificial Sequence
  tag sequence for base balance
aacacagccg

SEQ ID NO: 521 - DNA, 10 bp, Artificial Sequence
  tag sequence for base balance
tcataccaag

SEQ ID NO: 522 - DNA, 10 bp, Artificial Sequence
  tag sequence for base balance
gaagcttact

SEQ ID NO: 523 - DNA, 10 bp, Artificial Sequence
  tag sequence for base balance
gtcagtaggt

SEQ ID NO: 524 - DNA, 10 bp, Artificial Sequence
  tag sequence for base balance
ctgtgcgtag

SEQ ID NO: 525 - DNA, 10 bp, Artificial Sequence
  tag sequence for base balance
agtgaatgga

SEQ ID NO: 526 - DNA, 10 bp, Artificial Sequence
  tag sequence for base balance
tccacggttc

SEQ ID NO: 527 - DNA, 10 bp, Artificial Sequence
  tag sequence for base balance
aatctgcctc

SEQ ID NO: 528 - DNA, 10 bp, Artificial Sequence
  tag sequence for base balance
cggctaacca

SEQ ID NO: 529 - DNA, 10 bp, Artificial Sequence
  tag sequence for base balance
gacatacagt

SEQ ID NO: 530 - DNA, 10 bp, Artificial Sequence
  tag sequence for base balance
agaggcctca

SEQ ID NO: 531 - DNA, 10 bp, Artificial Sequence
  tag sequence for base balance
cctgatattg

SEQ ID NO: 532 - DNA, 10 bp, Artificial Sequence
  tag sequence for base balance
gtgctgaact

SEQ ID NO: 533 - DNA, 10 bp, Artificial Sequence
  tag sequence for base balance
cgatggtcag

SEQ ID NO: 534 - DNA, 10 bp, Artificial Sequence
  tag sequence for base balance
aatacagcgc

SEQ ID NO: 535 - DNA, 10 bp, Artificial Sequence
  tag sequence for base balance
tcgtcctgac

SEQ ID NO: 536 - DNA, 10 bp, Artificial Sequence
  tag sequence for base balance
ttccatggta

SEQ ID NO: 537 - DNA, 10 bp, Artificial Sequence
  tag sequence for base balance
cgttcgactg

SEQ ID NO: 538 - DNA, 10 bp, Artificial Sequence
  tag sequence for base balance
cgctacactc

SEQ ID NO: 539 - DNA, 10 bp, Artificial Sequence
  tag sequence for base balance
atagatcggt

SEQ ID NO: 540 - DNA, 10 bp, Artificial Sequence
  tag sequence for base balance
accagattca

SEQ ID NO: 541 - DNA, 10 bp, Artificial Sequence
  tag sequence for base balance
gatacggagg

SEQ ID NO: 542 - DNA, 10 bp, Artificial Sequence
  tag sequence for base balance
ttaggaggaa

SEQ ID NO: 543 - DNA, 10 bp, Artificial Sequence
  tag sequence for base balance
gcgcttctac

SEQ ID NO: 544 - DNA, 10 bp, Artificial Sequence
  tag sequence for base balance
tagctctact

SEQ ID NO: 545 - DNA, 10 bp, Artificial Sequence
  tag sequence for base balance
ccacctgctt

SEQ ID NO: 546 - DNA, 10 bp, Artificial Sequence
  tag sequence for base balance
cgtaggtctg

SEQ ID NO: 547 - DNA, 10 bp, Artificial Sequence
  tag sequence for base balance
tcttagtgac

SEQ ID NO: 548 - DNA, 10 bp, Artificial Sequence
  tag sequence for base balance
atcctagaac

SEQ ID NO: 549 - DNA, 10 bp, Artificial Sequence
  tag sequence for base balance
aggtgtaggt

SEQ ID NO: 550 - DNA, 10 bp, Artificial Sequence
  tag sequence for base balance
gtaaccatca

SEQ ID NO: 551 - DNA, 10 bp, Artificial Sequence
  tag sequence for base balance
taggtccaga

SEQ ID NO: 552 - DNA, 10 bp, Artificial Sequence
  tag sequence for base balance
gacgaactcg

SEQ ID NO: 553 - DNA, 10 bp, Artificial Sequence
  tag sequence for base balance
ccaacagatt

SEQ ID NO: 554 - DNA, 10 bp, Artificial Sequence
  tag sequence for base balance
cctctatctc

SEQ ID NO: 555 - DNA, 10 bp, Artificial Sequence
  tag sequence for base balance
gagtgtctca

SEQ ID NO: 556 - DNA, 10 bp, Artificial Sequence
  tag sequence for base balance
ttggcttaag

SEQ ID NO: 557 - DNA, 10 bp, Artificial Sequence
  tag sequence for base balance
agtcgcatgg

SEQ ID NO: 558 - DNA, 10 bp, Artificial Sequence
  tag sequence for base balance
atcttgcggc

SEQ ID NO: 559 - DNA, 10 bp, Artificial Sequence
  tag sequence for base balance
tgcaaggcct

SEQ ID NO: 560 - DNA, 10 bp, Artificial Sequence
  tag sequence for base balance
gaagacagaa

SEQ ID NO: 561 - DNA, 10 bp, Artificial Sequence
  tag sequence for base balance
acagactcat

SEQ ID NO: 562 - DNA, 10 bp, Artificial Sequence
  tag sequence for base balance
gagttgaggc

SEQ ID NO: 563 - DNA, 10 bp, Artificial Sequence
  tag sequence for base balance
gttctagacg

SEQ ID NO: 564 - DNA, 10 bp, Artificial Sequence
  tag sequence for base balance
agttcaggcg

SEQ ID NO: 565 - DNA, 10 bp, Artificial Sequence
  tag sequence for base balance
cagacgatga

SEQ ID NO: 566 - DNA, 10 bp, Artificial Sequence
  tag sequence for base balance
tccaacctat

SEQ ID NO: 567 - DNA, 10 bp, Artificial Sequence
  tag sequence for base balance
ttacgttctc

SEQ ID NO: 568 - DNA, 10 bp, Artificial Sequence
  tag sequence for base balance
cgcggtcata

SEQ ID NO: 569 - DNA, 10 bp, Artificial Sequence
  tag sequence for base balance
aatccttccg

SEQ ID NO: 570 - DNA, 10 bp, Artificial Sequence
  tag sequence for base balance
gaggattgaa

SEQ ID NO: 571 - DNA, 10 bp, Artificial Sequence
  tag sequence for base balance
atcggagtgc

SEQ ID NO: 572 - DNA, 10 bp, Artificial Sequence
  tag sequence for base balance
gcgttaagtg

SEQ ID NO: 573 - DNA, 10 bp, Artificial Sequence
  tag sequence for base balance
cctcggcaat

SEQ ID NO: 574 - DNA, 10 bp, Artificial Sequence
  tag sequence for base balance
ttaacggctt

SEQ ID NO: 575 - DNA, 10 bp, Artificial Sequence
  tag sequence for base balance
tgattccaca

SEQ ID NO: 576 - DNA, 10 bp, Artificial Sequence
  tag sequence for base balance
cgcaacatgc

SEQ ID NO: 577 - DNA, 10 bp, Artificial Sequence
  tag sequence for base balance
tcaatgaggt

SEQ ID NO: 578 - DNA, 10 bp, Artificial Sequence
  tag sequence for base balance
gtccaagctg

SEQ ID NO: 579 - DNA, 10 bp, Artificial Sequence
  tag sequence for base balance
gcgcactaag

SEQ ID NO: 580 - DNA, 10 bp, Artificial Sequence
  tag sequence for base balance
cggtgagtga

SEQ ID NO: 581 - DNA, 10 bp, Artificial Sequence
  tag sequence for base balance
tgaatccgac

SEQ ID NO: 582 - DNA, 10 bp, Artificial Sequence
  tag sequence for base balance
aatgctcact

SEQ ID NO: 583 - DNA, 10 bp, Artificial Sequence
  tag sequence for base balance
atcggttcca

SEQ ID NO: 584 - DNA, 10 bp, Artificial Sequence
  tag sequence for base balance
cattcgattc

SEQ ID NO: 585 - DNA, 10 bp, Artificial Sequence
  tag sequence for base balance
ttatgcctac

SEQ ID NO: 586 - DNA, 10 bp, Artificial Sequence
  tag sequence for base balance
atcctccgac

SEQ ID NO: 587 - DNA, 10 bp, Artificial Sequence
  tag sequence for base balance
cgcagatata

SEQ ID NO: 588 - DNA, 10 bp, Artificial Sequence
  tag sequence for base balance
acaacatgtg

SEQ ID NO: 589 - DNA, 10 bp, Artificial Sequence
  tag sequence for base balance
tcggatgagg

SEQ ID NO: 590 - DNA, 10 bp, Artificial Sequence
  tag sequence for base balance
cgtgcgatca

SEQ ID NO: 591 - DNA, 10 bp, Artificial Sequence
  tag sequence for base balance
gatcttacgt

SEQ ID NO: 592 - DNA, 10 bp, Artificial Sequence
  tag sequence for base balance
gagtaggcct

SEQ ID NO: 593 - DNA, 10 bp, Artificial Sequence
  tag sequence for base balance
aagagagaag

SEQ ID NO: 594 - DNA, 10 bp, Artificial Sequence
  tag sequence for base balance
gttctcacgg

SEQ ID NO: 595 - DNA, 10 bp, Artificial Sequence
  tag sequence for base balance
aagcggtgaa

SEQ ID NO: 596 - DNA, 10 bp, Artificial Sequence
  tag sequence for base balance
cgctcagtta

SEQ ID NO: 597 - DNA, 10 bp, Artificial Sequence
  tag sequence for base balance
ctagacactc

SEQ ID NO: 598 - DNA, 10 bp, Artificial Sequence
  tag sequence for base balance
gcttattgct

SEQ ID NO: 599 - DNA, 10 bp, Artificial Sequence
  tag sequence for base balance
tgcgttctgc

SEQ ID NO: 600 - DNA, 10 bp, Artificial Sequence
  tag sequence for base balance
tcaacgcact

SEQ ID NO: 601 - DNA, 10 bp, Artificial Sequence
  tag sequence for base balance
cttgcttaca

SEQ ID NO: 602 - DNA, 10 bp, Artificial Sequence
  tag sequence for base balance
ctcctcgcaa

SEQ ID NO: 603 - DNA, 10 bp, Artificial Sequence
  tag sequence for base balance
tctcagcctc

SEQ ID NO: 604 - DNA, 10 bp, Artificial Sequence
  tag sequence for base balance
gacggagtac

SEQ ID NO: 605 - DNA, 10 bp, Artificial Sequence
  tag sequence for base balance
acgtctatct

SEQ ID NO: 606 - DNA, 10 bp, Artificial Sequence
  tag sequence for base balance
gaatagagtg

SEQ ID NO: 607 - DNA, 10 bp, Artificial Sequence
  tag sequence for base balance
aggatacggt

SEQ ID NO: 608 - DNA, 10 bp, Artificial Sequence
  tag sequence for base balance
tgaagctagg

SEQ ID NO: 609 - DNA, 10 bp, Artificial Sequence
  tag sequence for base balance
aacctcgcac

SEQ ID NO: 610 - DNA, 10 bp, Artificial Sequence
  tag sequence for base balance
gatccggact

SEQ ID NO: 611 - DNA, 10 bp, Artificial Sequence
  tag sequence for base balance
gtgtctacag

SEQ ID NO: 612 - DNA, 10 bp, Artificial Sequence
  tag sequence for base balance
acggagaatc

SEQ ID NO: 613 - DNA, 10 bp, Artificial Sequence
  tag sequence for base balance
tgttacctca

SEQ ID NO: 614 - DNA, 10 bp, Artificial Sequence
  tag sequence for base balance
tcaatacgtg

SEQ ID NO: 615 - DNA, 10 bp, Artificial Sequence
  tag sequence for base balance
ctaagttggt

SEQ ID NO: 616 - DNA, 10 bp, Artificial Sequence
  tag sequence for base balance
cgcggattga

SEQ ID NO: 617 - DNA, 10 bp, Artificial Sequence
  tag sequence for base balance
acctcacata

SEQ ID NO: 618 - DNA, 10 bp, Artificial Sequence
  tag sequence for base balance
cggactgtct

SEQ ID NO: 619 - DNA, 10 bp, Artificial Sequence
  tag sequence for base balance
cgtggcagaa

SEQ ID NO: 620 - DNA, 10 bp, Artificial Sequence
  tag sequence for base balance
attcgaatgc

SEQ ID NO: 621 - DNA, 10 bp, Artificial Sequence
  tag sequence for base balance
taggttcaag

SEQ ID NO: 622 - DNA, 10 bp, Artificial Sequence
  tag sequence for base balance
gtccactctc

SEQ ID NO: 623 - DNA, 10 bp, Artificial Sequence
  tag sequence for base balance
gaatagtgct

SEQ ID NO: 624 - DNA, 10 bp, Artificial Sequence
  tag sequence for base balance
tcaatggcgg

SEQ ID NO: 625 - DNA, 10 bp, Artificial Sequence
  tag sequence for base balance
aagcatcctg

SEQ ID NO: 626 - DNA, 10 bp, Artificial Sequence
  tag sequence for base balance
gtggtgttca

SEQ ID NO: 627 - DNA, 10 bp, Artificial Sequence
  tag sequence for base balance
gtacaacgtt

SEQ ID NO: 628 - DNA, 10 bp, Artificial Sequence
  tag sequence for base balance
cctgcagcat

SEQ ID NO: 629 - DNA, 10 bp, Artificial Sequence
  tag sequence for base balance
tctatcgtac

SEQ ID NO: 630 - DNA, 10 bp, Artificial Sequence
  tag sequence for base balance
cactcgtagc

SEQ ID NO: 631 - DNA, 10 bp, Artificial Sequence
  tag sequence for base balance
tgcagcagca

SEQ ID NO: 632 - DNA, 10 bp, Artificial Sequence
  tag sequence for base balance
agatgtaagg

SEQ ID NO: 633 - DNA, 10 bp, Artificial Sequence
  tag sequence for base balance
gtgtaaccgc

SEQ ID NO: 634 - DNA, 10 bp, Artificial Sequence
  tag sequence for base balance
catcggaaga

SEQ ID NO: 635 - DNA, 10 bp, Artificial Sequence
  tag sequence for base balance
gaggaattac

SEQ ID NO: 636 - DNA, 10 bp, Artificial Sequence
  tag sequence for base balance
tgttcgctct

SEQ ID NO: 637 - DNA, 10 bp, Artificial Sequence
  tag sequence for base balance
accgtctata

SEQ ID NO: 638 - DNA, 10 bp, Artificial Sequence
  tag sequence for base balance
tgcctcagag

SEQ ID NO: 639 - DNA, 10 bp, Artificial Sequence
  tag sequence for base balance
acaagtgccg

SEQ ID NO: 640 - DNA, 10 bp, Artificial Sequence
  tag sequence for base balance
ctaactggtt

SEQ ID NO: 641 - DNA, 10 bp, Artificial Sequence
  tag sequence for base balance
cagaacgtgg

SEQ ID NO: 642 - DNA, 10 bp, Artificial Sequence
  tag sequence for base balance
gttcttctgt

SEQ ID NO: 643 - DNA, 10 bp, Artificial Sequence
  tag sequence for base balance
cggtgaagtc

SEQ ID NO: 644 - DNA, 10 bp, Artificial Sequence
  tag sequence for base balance
gtaagatgag

SEQ ID NO: 645 - DNA, 10 bp, Artificial Sequence
  tag sequence for base balance
tgccatcaca

SEQ ID NO: 646 - DNA, 10 bp, Artificial Sequence
  tag sequence for base balance
tcctcggata

SEQ ID NO: 647 - DNA, 10 bp, Artificial Sequence
  tag sequence for base balance
acagtgtcct

SEQ ID NO: 648 - DNA, 10 bp, Artificial Sequence
  tag sequence for base balance
aatgccacac

SEQ ID NO: 649 - DNA, 10 bp, Artificial Sequence
  tag sequence for base balance
gaccactcga

SEQ ID NO: 650 - DNA, 10 bp, Artificial Sequence
  tag sequence for base balance
atggacaaca

SEQ ID NO: 651 - DNA, 10 bp, Artificial Sequence
  tag sequence for base balance
aacctacggt

SEQ ID NO: 652 - DNA, 10 bp, Artificial Sequence
  tag sequence for base balance
tctaggattg

SEQ ID NO: 653 - DNA, 10 bp, Artificial Sequence
  tag sequence for base balance
cggattctcg

SEQ ID NO: 654 - DNA, 10 bp, Artificial Sequence
  tag sequence for base balance
cgatcttctc

SEQ ID NO: 655 - DNA, 10 bp, Artificial Sequence
  tag sequence for base balance
tcatcggaat

SEQ ID NO: 656 - DNA, 10 bp, Artificial Sequence
  tag sequence for base balance
gttggaggac

SEQ ID NO: 657 - DNA, 10 bp, Artificial Sequence
  tag sequence for base balance
acacatgcta

SEQ ID NO: 658 - DNA, 10 bp, Artificial Sequence
  tag sequence for base balance
ccttaggacg

SEQ ID NO: 659 - DNA, 10 bp, Artificial Sequence
  tag sequence for base balance
ctaaccaatc

SEQ ID NO: 660 - DNA, 10 bp, Artificial Sequence
  tag sequence for base balance
aacgcacgag

SEQ ID NO: 661 - DNA, 10 bp, Artificial Sequence
  tag sequence for base balance
gtcggttcac

SEQ ID NO: 662 - DNA, 10 bp, Artificial Sequence
  tag sequence for base balance
tggctcatgt

SEQ ID NO: 663 - DNA, 10 bp, Artificial Sequence
  tag sequence for base balance
tggtggttgt

SEQ ID NO: 664 - DNA, 10 bp, Artificial Sequence
  tag sequence for base balance
gatatacgca

SEQ ID NO: 665 - DNA, 10 bp, Artificial Sequence
  tag sequence for base balance
cacgaacact

SEQ ID NO: 666 - DNA, 10 bp, Artificial Sequence
  tag sequence for base balance
tgcgtgagca

SEQ ID NO: 667 - DNA, 10 bp, Artificial Sequence
  tag sequence for base balance
gtactgacga

SEQ ID NO: 668 - DNA, 10 bp, Artificial Sequence
  tag sequence for base balance
ccgtgagttc

SEQ ID NO: 669 - DNA, 10 bp, Artificial Sequence
  tag sequence for base balance
acttacttgg

SEQ ID NO: 670 - DNA, 10 bp, Artificial Sequence
  tag sequence for base balance
agaagctcat

SEQ ID NO: 671 - DNA, 10 bp, Artificial Sequence
  tag sequence for base balance
gttactggac

SEQ ID NO: 672 - DNA, 10 bp, Artificial Sequence
  tag sequence for base balance
tagcctcatg

SEQ ID NO: 673 - DNA, 10 bp, Artificial Sequence
  tag sequence for base balance
tgacaatgac

SEQ ID NO: 674 - DNA, 10 bp, Artificial Sequence
  tag sequence for base balance
aatcacctct

SEQ ID NO: 675 - DNA, 10 bp, Artificial Sequence
  tag sequence for base balance
aacagacctg

SEQ ID NO: 676 - DNA, 10 bp, Artificial Sequence
  tag sequence for base balance
gctagtgtgt

SEQ ID NO: 677 - DNA, 10 bp, Artificial Sequence
  tag sequence for base balance
gcggttgata

SEQ ID NO: 678 - DNA, 10 bp, Artificial Sequence
  tag sequence for base balance
ctagcgacac

SEQ ID NO: 679 - DNA, 10 bp, Artificial Sequence
  tag sequence for base balance
cggttgaacg

SEQ ID NO: 680 - DNA, 10 bp, Artificial Sequence
  tag sequence for base balance
ttctcctgga

SEQ ID NO: 681 - DNA, 10 bp, Artificial Sequence
  tag sequence for base balance
agttagctgg

SEQ ID NO: 682 - DNA, 10 bp, Artificial Sequence
  tag sequence for base balance
agtcctgtaa

SEQ ID NO: 683 - DNA, 10 bp, Artificial Sequence
  tag sequence for base balance
taaggccggt

SEQ ID NO: 684 - DNA, 10 bp, Artificial Sequence
  tag sequence for base balance
gccttatcct

SEQ ID NO: 685 - DNA, 10 bp, Artificial Sequence
  tag sequence for base balance
cagcattcaa

SEQ ID NO: 686 - DNA, 10 bp, Artificial Sequence
  tag sequence for base balance
tcgagcaatc

SEQ ID NO: 687 - DNA, 10 bp, Artificial Sequence
  tag sequence for base balance
gtaacgaacg

SEQ ID NO: 688 - DNA, 10 bp, Artificial Sequence
  tag sequence for base balance
ctcgtaggtc

SEQ ID NO: 689 - DNA, 10 bp, Artificial Sequence
  tag sequence for base balance
ctggattact

SEQ ID NO: 690 - DNA, 10 bp, Artificial Sequence
  tag sequence for base balance
gtatgttcct

SEQ ID NO: 691 - DNA, 10 bp, Artificial Sequence
  tag sequence for base balance
tgttcgcgac

SEQ ID NO: 692 - DNA, 10 bp, Artificial Sequence
  tag sequence for base balance
cacggaattg

SEQ ID NO: 693 - DNA, 10 bp, Artificial Sequence
  tag sequence for base balance
agcacaatgc

SEQ ID NO: 694 - DNA, 10 bp, Artificial Sequence
  tag sequence for base balance
acacaccgga

SEQ ID NO: 695 - DNA, 10 bp, Artificial Sequence
  tag sequence for base balance
tatctcgcta

SEQ ID NO: 696 - DNA, 10 bp, Artificial Sequence
  tag sequence for base balance
gcgatggaag

SEQ ID NO: 697 - DNA, 10 bp, Artificial Sequence
  tag sequence for base balance
taactcgtgg

SEQ ID NO: 698 - DNA, 10 bp, Artificial Sequence
  tag sequence for base balance
acaaccagta

SEQ ID NO: 699 - DNA, 10 bp, Artificial Sequence
  tag sequence for base balance
agcgtacgtc

SEQ ID NO: 700 - DNA, 10 bp, Artificial Sequence
  tag sequence for base balance
tcgactctgt

SEQ ID NO: 701 - DNA, 10 bp, Artificial Sequence
  tag sequence for base balance
ctgtatgcca

SEQ ID NO: 702 - DNA, 10 bp, Artificial Sequence
  tag sequence for base balance
gacgagacct

SEQ ID NO: 703 - DNA, 10 bp, Artificial Sequence
  tag sequence for base balance
cgttggtaac

SEQ ID NO: 704 - DNA, 10 bp, Artificial Sequence
  tag sequence for base balance
gttcgataag

SEQ ID NO: 705 - DNA, 10 bp, Artificial Sequence
  tag sequence for base balance
caagcgcgat

SEQ ID NO: 706 - DNA, 10 bp, Artificial Sequence
  tag sequence for base balance
gtgtgagtgc

SEQ ID NO: 707 - DNA, 10 bp, Artificial Sequence
  tag sequence for base balance
gcagcataat

SEQ ID NO: 708 - DNA, 10 bp, Artificial Sequence
  tag sequence for base balance
ttcttgtgca

SEQ ID NO: 709 - DNA, 10 bp, Artificial Sequence
  tag sequence for base balance
tggcacattg

SEQ ID NO: 710 - DNA, 10 bp, Artificial Sequence
  tag sequence for base balance
aacaatacgc

SEQ ID NO: 711 - DNA, 10 bp, Artificial Sequence
  tag sequence for base balance
cgtattgctg

SEQ ID NO: 712 - DNA, 10 bp, Artificial Sequence
  tag sequence for base balance
actcgccaca

SEQ ID NO: 713 - DNA, 10 bp, Artificial Sequence
  tag sequence for base balance
gctgcttggt

SEQ ID NO: 714 - DNA, 10 bp, Artificial Sequence
  tag sequence for base balance
ttgtggatac

SEQ ID NO: 715 - DNA, 10 bp, Artificial Sequence
  tag sequence for base balance
accaaggcga

SEQ ID NO: 716 - DNA, 10 bp, Artificial Sequence
  tag sequence for base balance
agaagaccta

SEQ ID NO: 717 - DNA, 10 bp, Artificial Sequence
  tag sequence for base balance
tagctctgtc

SEQ ID NO: 718 - DNA, 10 bp, Artificial Sequence
  tag sequence for base balance
cgacttctat

SEQ ID NO: 719 - DNA, 10 bp, Artificial Sequence
  tag sequence for base balance
ctctccaacg

SEQ ID NO: 720 - DNA, 10 bp, Artificial Sequence
  tag sequence for base balance
gatgaagacg

SEQ ID NO: 721 - DNA, 10 bp, Artificial Sequence
  tag sequence for base balance
tccagctcat

SEQ ID NO: 722 - DNA, 10 bp, Artificial Sequence
  tag sequence for base balance
accaagactc

SEQ ID NO: 723 - DNA, 10 bp, Artificial Sequence
  tag sequence for base balance
caactgcgca

SEQ ID NO: 724 - DNA, 10 bp, Artificial Sequence
  tag sequence for base balance
agtggatatc

SEQ ID NO: 725 - DNA, 10 bp, Artificial Sequence
  tag sequence for base balance
gtactaagag

SEQ ID NO: 726 - DNA, 10 bp, Artificial Sequence
  tag sequence for base balance
gtgtacgtcg

SEQ ID NO: 727 - DNA, 10 bp, Artificial Sequence
  tag sequence for base balance
cggtctctgt

SEQ ID NO: 728 - DNA, 10 bp, Artificial Sequence
  tag sequence for base balance
tatgctgaga

SEQ ID NO: 729 - DNA, 10 bp, Artificial Sequence
  tag sequence for base balance
aataggtagg

SEQ ID NO: 730 - DNA, 10 bp, Artificial Sequence
  tag sequence for base balance
agcttgcgct

SEQ ID NO: 731 - DNA, 10 bp, Artificial Sequence
  tag sequence for base balance
tggagccgat

SEQ ID NO: 732 - DNA, 10 bp, Artificial Sequence
  tag sequence for base balance
ccgcatacta

SEQ ID NO: 733 - DNA, 10 bp, Artificial Sequence
  tag sequence for base balance
ttcgatgacg

SEQ ID NO: 734 - DNA, 10 bp, Artificial Sequence
  tag sequence for base balance
gatccaatac

SEQ ID NO: 735 - DNA, 10 bp, Artificial Sequence
  tag sequence for base balance
gcattctcgc

SEQ ID NO: 736 - DNA, 10 bp, Artificial Sequence
  tag sequence for base balance
ctagcagtta

SEQ ID NO: 737 - DNA, 10 bp, Artificial Sequence
  tag sequence for base balance
cgttgacgct

SEQ ID NO: 738 - DNA, 10 bp, Artificial Sequence
  tag sequence for base balance
agtatatgcg

SEQ ID NO: 739 - DNA, 10 bp, Artificial Sequence
  tag sequence for base balance
acctccgcta

SEQ ID NO: 740 - DNA, 10 bp, Artificial Sequence
  tag sequence for base balance
caacacgaat

SEQ ID NO: 741 - DNA, 10 bp, Artificial Sequence
  tag sequence for base balance
ttgagtaagg

SEQ ID NO: 742 - DNA, 10 bp, Artificial Sequence
  tag sequence for base balance
gaagctctta

SEQ ID NO: 743 - DNA, 10 bp, Artificial Sequence
  tag sequence for base balance
tccgagatgc

SEQ ID NO: 744 - DNA, 10 bp, Artificial Sequence
  tag sequence for base balance
gtgctgtcac

SEQ ID NO: 745 - DNA, 10 bp, Artificial Sequence
  tag sequence for base balance
agcttccagc

SEQ ID NO: 746 - DNA, 10 bp, Artificial Sequence
  tag sequence for base balance
tgcctatcgc

SEQ ID NO: 747 - DNA, 10 bp, Artificial Sequence
  tag sequence for base balance
caatctcgcg

SEQ ID NO: 748 - DNA, 10 bp, Artificial Sequence
  tag sequence for base balance
cttcctacaa

SEQ ID NO: 749 - DNA, 10 bp, Artificial Sequence
  tag sequence for base balance
acgaggtact

SEQ ID NO: 750 - DNA, 10 bp, Artificial Sequence
  tag sequence for base balance
gatgaaggat

SEQ ID NO: 751 - DNA, 10 bp, Artificial Sequence
  tag sequence for base balance
tcgagcgtta

SEQ ID NO: 752 - DNA, 10 bp, Artificial Sequence
  tag sequence for base balance
gtagagattg

SEQ ID NO: 753 - DNA, 10 bp, Artificial Sequence
  tag sequence for base balance
acggctagag

SEQ ID NO: 754 - DNA, 10 bp, Artificial Sequence
  tag sequence for base balance
gctatagctt

SEQ ID NO: 755 - DNA, 10 bp, Artificial Sequence
  tag sequence for base balance
tgcgtcatgg

SEQ ID NO: 756 - DNA, 10 bp, Artificial Sequence
  tag sequence for base balance
ttccaacatc

SEQ ID NO: 757 - DNA, 10 bp, Artificial Sequence
  tag sequence for base balance
cggtgttgga

SEQ ID NO: 758 - DNA, 10 bp, Artificial Sequence
  tag sequence for base balance
gattgcgcct

SEQ ID NO: 759 - DNA, 10 bp, Artificial Sequence
  tag sequence for base balance
ataacgctca

SEQ ID NO: 760 - DNA, 10 bp, Artificial Sequence
  tag sequence for base balance
caacagtaac

SEQ ID NO: 761 - DNA, 10 bp, Artificial Sequence
  tag sequence for base balance
actggaggag

SEQ ID NO: 762 - DNA, 10 bp, Artificial Sequence
  tag sequence for base balance
gccggtaagt

SEQ ID NO: 763 - DNA, 10 bp, Artificial Sequence
  tag sequence for base balance
ctcacactta

SEQ ID NO: 764 - DNA, 10 bp, Artificial Sequence
  tag sequence for base balance
agacagtggc

SEQ ID NO: 765 - DNA, 10 bp, Artificial Sequence
  tag sequence for base balance
ctgatgtcct

SEQ ID NO: 766 - DNA, 10 bp, Artificial Sequence
  tag sequence for base balance
gagttcacaa

SEQ ID NO: 767 - DNA, 10 bp, Artificial Sequence
  tag sequence for base balance
tgttctcttc

SEQ ID NO: 768 - DNA, 10 bp, Artificial Sequence
  tag sequence for base balance
taacacgacg

SEQ ID NO: 769 - DNA, 31 bp, Artificial Sequence
  tag sequence for base balance
  misc_feature (1)..(31): solution 1 adapter 1
  misc_feature (1)..(1): 5phosphorylation
agtcggaggccaagcggtcttaggaagacaa

SEQ ID NO: 770 - DNA, 40 bp, Artificial Sequence
  tag sequence for base balance
  misc_feature (1)..(40): solution 1 adapter 2
  misc_feature (40)..(40): 3'-OH phosphorothioate
ttgtcttcctaacaggaacgacatggctacgatccgactt

SEQ ID NO: 771 - DNA, 64 bp, Artificial Sequence
  tag sequence for base balance
  misc_feature (1)..(64): solution 1 primer1
  misc_feature (1)..(1): 5'phosphorylation
  misc_feature (21)..(30): library tag sequence
ctctcagtacgtcagcagttnnnnnnnnnncaactccttggctcacagaacgacatggctacga

SEQ ID NO: 772 - DNA, 52 bp, Artificial Sequence
  tag sequence for base balance
  misc_feature (1)..(52): solution 1 primer2
  misc_feature (19)..(28): library tag sequence
gcatggcgaccttatcagnnnnnnnnnnttgtcttcctaagaccgcttggcc

SEQ ID NO: 773 - DNA, 35 bp, Artificial Sequence
  tag sequence for base balance
  misc_feature (1)..(35): solution 2 adapter 1
  misc_feature (1)..(1): 5'phosphorylation
agtcggaggccaagcggtcttaggaagacaatcag

SEQ ID NO: 774 - DNA, 59 bp, Artificial Sequence
  tag sequence for base balance
  misc_feature (1)..(59): solution 2 adapter 2
ctgattgtcttcctaagcaactccttggctcacagaacgacatggctacgatccgactt

SEQ ID NO: 775 - DNA, 51 bp, Artificial Sequence
  tag sequence for base balance
  misc_feature (1)..(51): solution 2 primer1
  misc_feature (1)..(1): 5'phosphorylation
  misc_feature (21)..(30): library tag sequence
ctctcagtacgtcagcagttnnnnnnnnnncaactccttggctcacagaac

SEQ ID NO: 776 - DNA, 50 bp, Artificial Sequence
  tag sequence for base balance
  misc_feature (1)..(50): solution 2 primer2
  misc_feature (19)..(28): library tag sequence
gcatggcgaccttatcagnnnnnnnnnnttgtcttcctaagaccgcttgg

SEQ ID NO: 777 - DNA, 10 bp, Artificial Sequence
  tag sequence for base balance
  misc_feature (1)..(10): MGI001tag1
atgcatctaa

SEQ ID NO: 778 - DNA, 10 bp, Artificial Sequence
  tag sequence for base balance
  misc_feature (1)..(10): MGI002tag1
agctctggac

SEQ ID NO: 779 - DNA, 10 bp, Artificial Sequence
  tag sequence for base balance
  misc_feature (1)..(10): MGI003tag1
ctatcacgtg

SEQ ID NO: 780 - DNA, 10 bp, Artificial Sequence
  tag sequence for base balance
  misc_feature (1)..(10): MGI004tag1
ggactagtgg

SEQ ID NO: 781 - DNA, 10 bp, Artificial Sequence
  tag sequence for base balance
  misc_feature (1)..(10): MGI005tag1
gccaagtcca

SEQ ID NO: 782 - DNA, 10 bp, Artificial Sequence
  tag sequence for base balance
  misc_feature (1)..(10): MGI006tag1
cctgtcaagc

SEQ ID NO: 783 - DNA, 10 bp, Artificial Sequence
  tag sequence for base balance
  misc_feature (1)..(10): MGI007tag1
tagaggtctt

SEQ ID NO: 784 - DNA, 10 bp, Artificial Sequence
  tag sequence for base balance
  misc_feature (1)..(10): MGI008tag1
tatggcaact

SEQ ID NO: 785 - DNA, 10 bp, Artificial Sequence
  tag sequence for base balance
  misc_feature (1)..(10): MGI001tag2
tagaggacaa

SEQ ID NO: 786 - DNA, 10 bp, Artificial Sequence
  tag sequence for base balance
  misc_feature (1)..(10): MGI002tag2
cctagcgaat

SEQ ID NO: 787 - DNA, 10 bp, Artificial Sequence
  tag sequence for base balance
  misc_feature (1)..(10): MGI003tag2
gtagtcatcg

SEQ ID NO: 788 - DNA, 10 bp, Artificial Sequence
  tag sequence for base balance
  misc_feature (1)..(10): MGI004tag2
gctgagctgt

SEQ ID NO: 789 - DNA, 10 bp, Artificial Sequence
  tag sequence for base balance
  misc_feature (1)..(10): MGI005tag2
aacctagata

SEQ ID NO: 790 - DNA, 10 bp, Artificial Sequence
  tag sequence for base balance
  misc_feature (1)..(10): MGI006tag2
ttgccatctc

SEQ ID NO: 791 - DNA, 10 bp, Artificial Sequence
  tag sequence for base balance
  misc_feature (1)..(10): MGI007tag2
agatcttgcg

SEQ ID NO: 792 - DNA, 10 bp, Artificial Sequence
  tag sequence for base balance
  misc_feature (1)..(10): MGI008tag2
cgctatcggc

SEQ ID NO: 793 - DNA, 20 bp, Artificial Sequence
  tag sequence for base balance
  misc_feature (1)..(20): universial amplification sequence
  misc_feature (1)..(1): 5'
ctctcagtacgtcagcagtt

SEQ ID NO: 794 - DNA, 34 bp, Artificial Sequence
  tag sequence for base balance
  misc_feature (1)..(34): universial primer
caactccttggctcacagaacgacatggctacga

SEQ ID NO: 795 - DNA, 18 bp, Artificial Sequence
  tag sequence for base balance
  misc_feature (1)..(18): universial primer
gcatggcgaccttatcag

SEQ ID NO: 796 - DNA, 24 bp, Artificial Sequence
  tag sequence for base balance
  misc_feature (1)..(24): universial primer
ttgtcttcctaagaccgcttggcc

SEQ ID NO: 797 - DNA, 21 bp, Artificial Sequence
  tag sequence for base balance
  misc_feature (1)..(21): universial amplification sequence
caactccttggctcacagaac

SEQ ID NO: 798 - DNA, 22 bp, Artificial Sequence
  tag sequence for base balance
  misc_feature (1)..(22): universial amplification sequence
ttgtcttcctaagaccgcttgg